European Patent Specification EP 3 415 167 B1, published May 29, 2024. Title: INTRATHECAL DELIVERY OF RECOMBINANT ADENO-ASSOCIATED VIRUS 9. Applicant: NATIONWIDE CHILDREN'S HOSPITAL, INC. OHIO STATE INNOVATION FOUNDATION. Application 13747755.0. The sequence listing filed with the application follows.

SEQUENCE LISTING (1 sequence)

SEQ ID NO: 1 - DNA, 6042 bp, adeno-associated virus 9
  misc_feature (980)..(3336): Vector genome insert
  misc_feature (980)..(1085): Mutated ITR
  misc_feature (1132)..(1411): CMV enhancer
  misc_feature (1418)..(1687): Chicken beta-Actin promoter
  misc_feature (1753)..(1812): Modified SV40 late 16s intron
  misc_feature (1753)..(1783): SV40 late 19s intron
  misc_feature (1982)..(2866): hSMN
  misc_feature (2970)..(3116): BGHpA
  misc_feature (3196)..(3336): ITR
gcccaatacgcaaaccgcctctccccgcgcgttggccgattcattaatgcagctggcgtaatagcgaagaggcccgcaccgatcgcccttcccaacagttgcgcagcctgaatggcgaatggcgattccgttgcaatggctggcggtaatattgttctggatattaccagcaaggccgatagtttgagttcttctactcaggcaagtgatgttattactaatcaaagaagtattgcgacaacggttaatttgcgtgatggacagactcttttactcggtggcctcactgattataaaaacacttctcaggattctggcgtaccgttcctgtctaaaatccctttaatcggcctcctgtttagctcccgctctgattctaacgaggaaagcacgttatacgtgctcgtcaaagcaaccatagtacgcgccctgtagcggcgcattaagcgcggcgggtgtggtggttacgcgcagcgtgaccgctacacttgccagcgccctagcgcccgctcctttcgctttcttcccttcctttctcgccacgttcgccggctttccccgtcaagctctaaatcgggggctccctttagggttccgatttagtgctttacggcacctcgaccccaaaaaacttgattagggtgatggttcacgtagtgggccatcgccctgatagacggtttttcgccctttgacgttggagtccacgttctttaatagtggactcttgttccaaactggaacaacactcaaccctatctcggtctattcttttgatttataagggattttgccgatttcggcctattggttaaaaaatgagctgatttaacaaaaatttaacgcgaattttaacaaaatattaacgcttacaatttaaatatttgcttatacaatcttcctgtttttggggcttttctgattatcaaccggggtacatatgattgacatgctagttttacgattaccgttcatcgccctgcgcgctcgctcgctcactgaggccgcccgggcaaagcccgggcgtcgggcgacctttggtcgcccggcctcagtgagcgagcgagcgcgcagagagggagtggaattcacgcgtggatctgaattcaattcacgcgtggtacctctggtcgttacataacttacggtaaatggcccgcctggctgaccgcccaacgacccccgcccattgacgtcaataatgacgtatgttcccatagtaacgccaatagggactttccattgacgtcaatgggtggagtatttacggtaaactgcccacttggcagtacatcaagtgtatcatatgccaagtacgccccctattgacgtcaatgacggtaaatggcccgcctggcattatgcccagtacatgaccttatgggactttcctacttggcagtacatctactcgaggccacgttctgcttcactctccccatctcccccccctccccacccccaattttgtatttatttattttttaattattttgtgcagcgatgggggcggggggggggggggggcgcgcgccaggcggggcggggcggggcgaggggcggggcggggcgaggcggagaggtgcggcggcagccaatcagagcggcgcgctccgaaagtttccttttatggcgaggcggcggcggcggcggccctataaaaagcgaagcgcgcggcgggcgggagcgggatcagccaccgcggtggcggcctagagtcgacgaggaactgaaaaaccagaaagttaactggtaagtttagtctttttgtcttttatttcaggtcccggatccggtggtggtgcaaatcaaagaactgctcctcagtggatgttgcctttacttctaggcctgtacggaagtgttacttctgctctaaaagctgcggaattgtacccgcggccgatccaccggtccggaattcccgggatatcgtcgacccacgcgtccgggccccacgctgcgcacccgcgggtttgctatggcgatgagcagcggcggcagtggtggcggcgtcccggagcaggaggattccgtgctgttccggcgcggcacaggccagagcgatgattctgacatttgggatgatacagcactgataaaagcatatgataaagctgtggcttcatttaagcatgctctaaagaatggtgacatttgtgaaacttcgggtaaaccaaaaaccacacctaaaagaaaacctgctaagaagaataaaagccaaaagaagaatactgcagcttccttacaacagtggaaagttggggacaaatgttctgccatttggtcagaagacggttgcatttacccagctaccattgcttcaattgattttaagagagaaacctgtgttgtggtttacactggatatggaaatagagaggagcaaaatctgtccgatctactttccccaatctgtgaagtagctaataatatagaacagaatgctcaagagaatgaaaatgaaagccaagtttcaacagatgaaagtgagaactccaggtctcctggaaataaatcagataacatcaagcccaaatctgctccatggaactcttttctccctccaccaccccccatgccagggccaagactgggaccaggaaagccaggtctaaaattcaatggcccaccaccgccaccgccaccaccaccaccccacttactatcatgctggctgcctccatttccttctggaccaccaataattcccccaccacctcccatatgtccagattctcttgatgatgctgatgctttgggaagtatgttaatttcatggtacatgagtggctatcatactggctattatatgggttttagacaaaatcaaaaagaaggaaggtgctcacattccttaaattaaggagaaatgctggcatagagcagcactaaatgacaccactaaagaaacgatcagacagatctagaaagcttatcgataccgtcgactagagctcgctgatcagcctcgactgtgccttctagttgccagccatctgttgtttgcccctcccccgtgccttccttgaccctggaaggtgccactcccactgtcctttcctaataaaatgaggaaattgcatcgcattgtctgagtaggtgtcattctattctggggggtggggtggggcaggacagcaagggggaggattgggaagacaatagcaggcatgctggggagagatcgatctgaggaacccctagtgatggagttggccactccctctctgcgcgctcgctcgctcactgaggccgggcgaccaaaggtcgcccgacgcccgggctttgcccgggcggcctcagtgagcgagcgagcgcgcagagagggagtggcccccccccccccccccccggcgattctcttgtttgctccagactctcaggcaatgacctgatagcctttgtagagacctctcaaaaatagctaccctctccggcatgaatttatcagctagaacggttgaatatcatattgatggtgatttgactgtctccggcctttctcacccgtttgaatctttacctacacattactcaggcattgcatttaaaatatatgagggttctaaaaatttttatccttgcgttgaaataaaggcttctcccgcaaaagtattacagggtcataatgtttttggtacaaccgatttagctttatgctctgaggctttattgcttaattttgctaattctttgccttgcctgtatgatttattggatgttggaatcgcctgatgcggtattttctccttacgcatctgtgcggtatttcacaccgcatatggtgcactctcagtacaatctgctctgatgccgcatagttaagccagccccgacacccgccaacactatggtgcactctcagtacaatctgctctgatgccgcatagttaagccagccccgacacccgccaacacccgctgacgcgccctgacgggcttgtctgctcccggcatccgcttacagacaagctgtgaccgtctccgggagctgcatgtgtcagaggttttcaccgtcatcaccgaaacgcgcgagacgaaagggcctcgtgatacgcctatttttataggttaatgtcatgataataatggtttcttagacgtcaggtggcacttttcggggaaatgtgcgcggaacccctatttgtttatttttctaaatacattcaaatatgtatccgctcatgagacaataaccctgataaatgcttcaataatattgaaaaaggaagagtatgagtattcaacatttccgtgtcgcccttattcccttttttgcggcattttgccttcctgtttttgctcacccagaaacgctggtgaaagtaaaagatgctgaagatcagttgggtgcacgagtgggttacatcgaactggatctcaacagcggtaagatccttgagagttttcgccccgaagaacgttttccaatgatgagcacttttaaagttctgctatgtggcgcggtattatcccgtattgacgccgggcaagagcaactcggtcgccgcatacactattctcagaatgacttggttgagtactcaccagtcacagaaaagcatcttacggatggcatgacagtaagagaattatgcagtgctgccataaccatgagtgataacactgcggccaacttacttctgacaacgatcggaggaccgaaggagctaaccgcttttttgcacaacatgggggatcatgtaactcgccttgatcgttgggaaccggagctgaatgaagccataccaaacgacgagcgtgacaccacgatgcctgtagcaatggcaacaacgttgcgcaaactattaactggcgaactacttactctagcttcccggcaacaattaatagactggatggaggcggataaagttgcaggaccacttctgcgctcggcccttccggctggctggtttattgctgataaatctggagccggtgagcgtgggtctcgcggtatcattgcagcactggggccagatggtaagccctcccgtatcgtagttatctacacgacggggagtcaggcaactatggatgaacgaaatagacagatcgctgagataggtgcctcactgattaagcattggtaactgtcagaccaagtttactcatatatactttagattgatttaaaacttcatttttaatttaaaaggatctaggtgaagatcctttttgataatctcatgaccaaaatcccttaacgtgagttttcgttccactgagcgtcagaccccgtagaaaagatcaaaggatcttcttgagatcctttttttctgcgcgtaatctgctgcttgcaaacaaaaaaaccaccgctaccagcggtggtttgtttgccggatcaagagctaccaactctttttccgaaggtaactggcttcagcagagcgcagataccaaatactgttcttctagtgtagccgtagttaggccaccacttcaagaactctgtagcaccgcctacatacctcgctctgctaatcctgttaccagtggctgctgccagtggcgataagtcgtgtcttaccgggttggactcaagacgatagttaccggataaggcgcagcggtcgggctgaacggggggttcgtgcacacagcccagcttggagcgaacgacctacaccgaactgagatacctacagcgtgagctatgagaaagcgccacgcttcccgaagggagaaaggcggacaggtatccggtaagcggcagggtcggaacaggagagcgcacgagggagcttccagggggaaacgcctggtatctttatagtcctgtcgggtttcgccacctctgacttgagcgtcgatttttgtgatgctcgtcaggggggcggagcctatggaaaaacgccagcaacgcggcctttttacggttcctggccttttgctggccttttgctcacatgttctttcctgcgttatcccctgattctgtggataaccgtattaccgcctttgagtgagctgataccgctcgccgcagccgaacgaccgagcgcagcgagtcagtgagcgaggaagcggaagagc